European Patent Application EP 4 403 573 A1, published July 24, 2024. Title: PHARMACEUTICAL COMPOSITION COMPRISING ANTI-PVRIG/TIGIT BISPECIFIC ANTIBODY. Applicant: JIANGSU HENGRUI PHARMACEUTICALS CO., LTD. Application WO PCT/CN2022/118942, filed September 15, 2022. The sequence listing filed with the application follows.

SEQUENCE LISTING (165 sequences)

SEQ ID NO: 1 - protein, 137 aa, synthetic construct
  REGION 1..137: note = his1PVRIG (cyno-PVRIG-his)
TPEVWVQVQMEATELSSFTVHCGFLGPGSISLVTVSWGGPDGAGGTKLAVLHPELGTRQWAPARQARWETQSSISLALEDSGASSPFANTTFCCKFASFPEGSWESCGSLPPSSDPGLSAPPTPVPILRADHHHHHH

SEQ ID NO: 2 - protein, 121 aa, synthetic construct
  REGION 1..121: note = 20-HCVR
DVQLVESGGGSVQAGGSLRLSCVASRYTSRTDCMGWFRQAPGKEHEGVAHIDSDGIPRYVDSVKGRFTISQDHAKNTLYLQMNSLKPEDSATYYCVVGFKFDDDYCAPNDWGQGTQVTVSS

SEQ ID NO: 3 - protein, 121 aa, synthetic construct
  REGION 1..121: note = 30-HCVR
HVQLVESGGGSVQAGGSLRLSCEASGYSYSGDCMGWFRRAPGKERDEGVATIDNAGRIKYADSVKGRFTISHGNGKYILYLQMNSLKPEDTDMYYCAAGWTFGGNCSPADWGQGTQVTVSS

SEQ ID NO: 4 - protein, 123 aa, synthetic construct
  REGION 1..123: note = 38-HCVR
QVQLVESGGGSVQAGGSLRLSCAASPSTYGPSDMAWFRQAPGKQREGVATISAAGRLTYYTDSVRGRFTISRDNAKNTMYLQMNSLKPEDTAMYYCAADFAGGSSLFADYKYWGQGTQVTVSS

SEQ ID NO: 5 - protein, 120 aa, synthetic construct
  REGION 1..120: note = 39-HCVR
QVQLVESGGGSVQAGGSLRLSCAASRYTSRTDCMGWFRQAPGKEREGVAHIDSDGIPRYVESVKGRFTISQDHAKNTLYLQMNSLKPEDSATYYCVVGFKFGDYCAPNDWGQGTQVTVSS

SEQ ID NO: 6 - protein, 127 aa, synthetic construct
  REGION 1..127: note = 151-HCVR
HVQLVESGGGSVQAGGSLRLSCVASASGFTYRPYCMAWFRQAPGKEREAVAGIDIFGGTTYADSVKGRFTASRDNAGFSLFLQMNDLKPEDTAMYYCAAGDSPDGRCPPLGQGLNYWGQGTQVTVSS

SEQ ID NO: 7 - protein, 5 aa, synthetic construct
  REGION 1..5: note = 20 HCDR1
TDCMG

SEQ ID NO: 8 - protein, 16 aa, synthetic construct
  REGION 1..16: note = 20 HCDR2
HIDSDGIPRYVDSVKG

SEQ ID NO: 9 - protein, 13 aa, synthetic construct
  REGION 1..13: note = 20 HCDR3
GFKFDDDYCAPND

SEQ ID NO: 10 - protein, 5 aa, synthetic construct
  REGION 1..5: note = 30 HCDR1
GDCMG

SEQ ID NO: 11 - protein, 16 aa, synthetic construct
  REGION 1..16: note = 30 HCDR2
TIDNAGRIKYADSVKG

SEQ ID NO: 12 - protein, 12 aa, synthetic construct
  REGION 1..12: note = 30 HCDR3
GWTFGGNCSPAD

SEQ ID NO: 13 - protein, 5 aa, synthetic construct
  REGION 1..5: note = 38 HCDR1
PSDMA

SEQ ID NO: 14 - protein, 17 aa, synthetic construct
  REGION 1..17: note = 38 HCDR2
TISAAGRLTYYTDSVRG

SEQ ID NO: 15 - protein, 14 aa, synthetic construct
  REGION 1..14: note = 38 HCDR3
DFAGGSSLFADYKY

SEQ ID NO: 16 - protein, 5 aa, synthetic construct
  REGION 1..5: note = 39 HCDR1
TDCMG

SEQ ID NO: 17 - protein, 16 aa, synthetic construct
  REGION 1..16: note = 39 HCDR2
HIDSDGIPRYVESVKG

SEQ ID NO: 18 - protein, 12 aa, synthetic construct
  REGION 1..12: note = 39 HCDR3
GFKFGDYCAPND

SEQ ID NO: 19 - protein, 7 aa, synthetic construct
  REGION 1..7: note = 151 HCDR1
YRPYCMA

SEQ ID NO: 20 - protein, 16 aa, synthetic construct
  REGION 1..16: note = 151 HCDR2
GIDIFGGTTYADSVKG

SEQ ID NO: 21 - protein, 17 aa, synthetic construct
  REGION 1..17: note = 151 HCDR3
GDSPDGRCPPLGQGLNY

SEQ ID NO: 22 - protein, 7 aa, synthetic construct
  REGION 1..7: note = 20 HCDR1 CHO
RYTSRTD

SEQ ID NO: 23 - protein, 5 aa, synthetic construct
  REGION 1..5: note = 20 HCDR2 CHO
DSDGI

SEQ ID NO: 24 - protein, 13 aa, synthetic construct
  REGION 1..13: note = 20 HCDR3 CHO
GFKFDDDYCAPND

SEQ ID NO: 25 - protein, 7 aa, synthetic construct
  REGION 1..7: note = 30 HCDR1 CHO
GYSYSGD

SEQ ID NO: 26 - protein, 5 aa, synthetic construct
  REGION 1..5: note = 30 HCDR2 CHO
DNAGR

SEQ ID NO: 27 - protein, 12 aa, synthetic construct
  REGION 1..12: note = 30 HCDR3 CHO
GWTFGGNCSPAD

SEQ ID NO: 28 - protein, 7 aa, synthetic construct
  REGION 1..7: note = 38 HCDR1 CHO
PSTYGPS

SEQ ID NO: 29 - protein, 6 aa, synthetic construct
  REGION 1..6: note = 38 HCDR2 CHO
SAAGRL

SEQ ID NO: 30 - protein, 14 aa, synthetic construct
  REGION 1..14: note = 38 HCDR3 CHO
DFAGGSSLFADYKY

SEQ ID NO: 31 - protein, 7 aa, synthetic construct
  REGION 1..7: note = 39 HCDR1 CHO
RYTSRTD

SEQ ID NO: 32 - protein, 5 aa, synthetic construct
  REGION 1..5: note = 39 HCDR2 CHO
DSDGI

SEQ ID NO: 33 - protein, 12 aa, synthetic construct
  REGION 1..12: note = 39 HCDR3 CHO
GFKFGDYCAPND

SEQ ID NO: 34 - protein, 9 aa, synthetic construct
  REGION 1..9: note = 151 HCDR1 CHO
ASGFTYRPY

SEQ ID NO: 35 - protein, 5 aa, synthetic construct
  REGION 1..5: note = 151 HCDR2 CHO
DIFGG

SEQ ID NO: 36 - protein, 17 aa, synthetic construct
  REGION 1..17: note = 151 HCDR3 CHO
GDSPDGRCPPLGQGLNY

SEQ ID NO: 37 - protein, 8 aa, synthetic construct
  REGION 1..8: note = 20 HCDR1 IMGT
RYTSRTDC

SEQ ID NO: 38 - protein, 7 aa, synthetic construct
  REGION 1..7: note = 20 HCDR2 IMGT
IDSDGIP

SEQ ID NO: 39 - protein, 15 aa, synthetic construct
  REGION 1..15: note = 20 HCDR3 IMGT
VVGFKFDDDYCAPND

SEQ ID NO: 40 - protein, 8 aa, synthetic construct
  REGION 1..8: note = 30 HCDR1 IMGT
GYSYSGDC

SEQ ID NO: 41 - protein, 7 aa, synthetic construct
  REGION 1..7: note = 30 HCDR2 IMGT
IDNAGRI

SEQ ID NO: 42 - protein, 14 aa, synthetic construct
  REGION 1..14: note = 30 HCDR3 IMGT
AAGWTFGGNCSPAD

SEQ ID NO: 43 - protein, 8 aa, synthetic construct
  REGION 1..8: note = 38 HCDR1 IMGT
PSTYGPSD

SEQ ID NO: 44 - protein, 8 aa, synthetic construct
  REGION 1..8: note = 38 HCDR2 IMGT
ISAAGRLT

SEQ ID NO: 45 - protein, 16 aa, synthetic construct
  REGION 1..16: note = 38 HCDR3 IMGT
AADFAGGSSLFADYKY

SEQ ID NO: 46 - protein, 8 aa, synthetic construct
  REGION 1..8: note = 39 HCDR1 IMGT
RYTSRTDC

SEQ ID NO: 47 - protein, 7 aa, synthetic construct
  REGION 1..7: note = 39 HCDR2 IMGT
IDSDGIP

SEQ ID NO: 48 - protein, 14 aa, synthetic construct
  REGION 1..14: note = 39 HCDR3 IMGT
VVGFKFGDYCAPND

SEQ ID NO: 49 - protein, 10 aa, synthetic construct
  REGION 1..10: note = 151 HCDR1 IMGT
ASGFTYRPYC

SEQ ID NO: 50 - protein, 7 aa, synthetic construct
  REGION 1..7: note = 151 HCDR2 IMGT
IDIFGGT

SEQ ID NO: 51 - protein, 19 aa, synthetic construct
  REGION 1..19: note = 151 HCDR3 IMGT
AAGDSPDGRCPPLGQGLNY

SEQ ID NO: 52 - protein, 10 aa, synthetic construct
  REGION 1..10: note = 20 HCDR1 ABM
RYTSRTDCMG

SEQ ID NO: 53 - protein, 9 aa, synthetic construct
  REGION 1..9: note = 20 HCDR2 ABM
HIDSDGIPR

SEQ ID NO: 54 - protein, 13 aa, synthetic construct
  REGION 1..13: note = 20 HCDR3 ABM
GFKFDDDYCAPND

SEQ ID NO: 55 - protein, 10 aa, synthetic construct
  REGION 1..10: note = 30 HCDR1 ABM
GYSYSGDCMG

SEQ ID NO: 56 - protein, 9 aa, synthetic construct
  REGION 1..9: note = 30 HCDR2 ABM
TIDNAGRIK

SEQ ID NO: 57 - protein, 12 aa, synthetic construct
  REGION 1..12: note = 30 HCDR3 ABM
GWTFGGNCSPAD

SEQ ID NO: 58 - protein, 10 aa, synthetic construct
  REGION 1..10: note = 38 HCDR1 ABM
PSTYGPSDMA

SEQ ID NO: 59 - protein, 10 aa, synthetic construct
  REGION 1..10: note = 38 HCDR2 ABM
TISAAGRLTY

SEQ ID NO: 60 - protein, 14 aa, synthetic construct
  REGION 1..14: note = 38 HCDR3 ABM
DFAGGSSLFADYKY

SEQ ID NO: 61 - protein, 10 aa, synthetic construct
  REGION 1..10: note = 39 HCDR1 ABM
RYTSRTDCMG

SEQ ID NO: 62 - protein, 9 aa, synthetic construct
  REGION 1..9: note = 39 HCDR2 ABM
HIDSDGIPR

SEQ ID NO: 63 - protein, 12 aa, synthetic construct
  REGION 1..12: note = 39 HCDR3 ABM
GFKFGDYCAPND

SEQ ID NO: 64 - protein, 12 aa, synthetic construct
  REGION 1..12: note = 151 HCDR1 ABM
ASGFTYRPYCMA

SEQ ID NO: 65 - protein, 9 aa, synthetic construct
  REGION 1..9: note = 151 HCDR2 ABM
GIDIFGGTT

SEQ ID NO: 66 - protein, 17 aa, synthetic construct
  REGION 1..17: note = 151 HCDR3 ABM
GDSPDGRCPPLGQGLNY

SEQ ID NO: 67 - protein, 350 aa, synthetic construct
  REGION 1..350: note = 20 HC
DVQLVESGGGSVQAGGSLRLSCVASRYTSRTDCMGWFRQAPGKEHEGVAHIDSDGIPRYVDSVKGRFTISQDHAKNTLYLQMNSLKPEDSATYYCVVGFKFDDDYCAPNDWGQGTQVTVSSESKYGPPCPPCPAPEAAGGPSVFLFPPKPKDTLMISRTPEVTCVVVDVSQEDPEVQFNWYVDGVEVHNAKTKPREEQFNSTYRVVSVLTVLHQDWLNGKEYKCKVSNKGLPSSIEKTISKAKGQPREPQVYTLPPSQEEMTKNQVSLTCLVKGFYPSDIAVEWESNGQPENNYKTTPPVLDSDGSFFLYSRLTVDKSRWQEGNVFSCSVMHEALHNHYTQKSLSLSLGA

SEQ ID NO: 68 - protein, 350 aa, synthetic construct
  REGION 1..350: note = 30 HC
HVQLVESGGGSVQAGGSLRLSCEASGYSYSGDCMGWFRRAPGKERDEGVATIDNAGRIKYADSVKGRFTISHGNGKYILYLQMNSLKPEDTDMYYCAAGWTFGGNCSPADWGQGTQVTVSSESKYGPPCPPCPAPEAAGGPSVFLFPPKPKDTLMISRTPEVTCVVVDVSQEDPEVQFNWYVDGVEVHNAKTKPREEQFNSTYRVVSVLTVLHQDWLNGKEYKCKVSNKGLPSSIEKTISKAKGQPREPQVYTLPPSQEEMTKNQVSLTCLVKGFYPSDIAVEWESNGQPENNYKTTPPVLDSDGSFFLYSRLTVDKSRWQEGNVFSCSVMHEALHNHYTQKSLSLSLGA

SEQ ID NO: 69 - protein, 352 aa, synthetic construct
  REGION 1..352: note = 38 HC
QVQLVESGGGSVQAGGSLRLSCAASPSTYGPSDMAWFRQAPGKQREGVATISAAGRLTYYTDSVRGRFTISRDNAKNTMYLQMNSLKPEDTAMYYCAADFAGGSSLFADYKYWGQGTQVTVSSESKYGPPCPPCPAPEAAGGPSVFLFPPKPKDTLMISRTPEVTCVVVDVSQEDPEVQFNWYVDGVEVHNAKTKPREEQFNSTYRVVSVLTVLHQDWLNGKEYKCKVSNKGLPSSIEKTISKAKGQPREPQVYTLPPSQEEMTKNQVSLTCLVKGFYPSDIAVEWESNGQPENNYKTTPPVLDSDGSFFLYSRLTVDKSRWQEGNVFSCSVMHEALHNHYTQKSLSLSLGA

SEQ ID NO: 70 - protein, 349 aa, synthetic construct
  REGION 1..349: note = 39 HC
QVQLVESGGGSVQAGGSLRLSCAASRYTSRTDCMGWFRQAPGKEREGVAHIDSDGIPRYVESVKGRFTISQDHAKNTLYLQMNSLKPEDSATYYCVVGFKFGDYCAPNDWGQGTQVTVSSESKYGPPCPPCPAPEAAGGPSVFLFPPKPKDTLMISRTPEVTCVVVDVSQEDPEVQFNWYVDGVEVHNAKTKPREEQFNSTYRVVSVLTVLHQDWLNGKEYKCKVSNKGLPSSIEKTISKAKGQPREPQVYTLPPSQEEMTKNQVSLTCLVKGFYPSDIAVEWESNGQPENNYKTTPPVLDSDGSFFLYSRLTVDKSRWQEGNVFSCSVMHEALHNHYTQKSLSLSLGA

SEQ ID NO: 71 - protein, 356 aa, synthetic construct
  REGION 1..356: note = 151 HC
HVQLVESGGGSVQAGGSLRLSCVASASGFTYRPYCMAWFRQAPGKEREAVAGIDIFGGTTYADSVKGRFTASRDNAGFSLFLQMNDLKPEDTAMYYCAAGDSPDGRCPPLGQGLNYWGQGTQVTVSSESKYGPPCPPCPAPEAAGGPSVFLFPPKPKDTLMISRTPEVTCVVVDVSQEDPEVQFNWYVDGVEVHNAKTKPREEQFNSTYRVVSVLTVLHQDWLNGKEYKCKVSNKGLPSSIEKTISKAKGQPREPQVYTLPPSQEEMTKNQVSLTCLVKGFYPSDIAVEWESNGQPENNYKTTPPVLDSDGSFFLYSRLTVDKSRWQEGNVFSCSVMHEALHNHYTQKSLSLSLGA

SEQ ID NO: 72 - protein, 449 aa, synthetic construct
  REGION 1..449: note = tab5 HC
EVQLVESGGGVVKPGGSLRLSCAASGFTFGTSSMNWVRQAPGKGLEWVAVISFDGTEIHYADSVKGRFTISRDNSKSTVFLQMNSLRPDDTALYYCAKGSGNIYFYSGMDVWGQGTTVTVSSASTKGPSVFPLAPCSRSTSESTAALGCLVKDYFPEPVTVSWNSGALTSGVHTFPAVLQSSGLYSLSSVVTVPSSSLGTKTYTCNVDHKPSNTKVDKRVESKYGPPCPPCPAPEAAGGPSVFLFPPKPKDTLMISRTPEVTCVVVDVSQEDPEVQFNWYVDGVEVHNAKTKPREEQFNSTYRVVSVLTVLHQDWLNGKEYKCKVSNKGLPSSIEKTISKAKGQPREPQVYTLPPSQEEMTKNQVSLTCLVKGFYPSDIAVEWESNGQPENNYKTTPPVLDSDGSFFLYSRLTVDKSRWQEGNVFSCSVMHEALHNHYTQKSLSLSLGA

SEQ ID NO: 73 - protein, 214 aa, synthetic construct
  REGION 1..214: note = tab5 LC
DIQMTQSPSTLSASVGDRVTITCRAGQSISGWLAWFQQKPGKAPNLLIYETSTLESGVPSRFSGSGSGTEYTLTISSLQPDDFATYYCQQYYSYPLTFGQGTKVEIKRTVAAPSVFIFPPSDEQLKSGTASVVCLLNNFYPREAKVQWKVDNALQSGNSQESVTEQDSKDSTYSLSSTLTLSKADYEKHKVYACEVTHQGLSSPVTKSFNRGEC

SEQ ID NO: 74 - protein, 98 aa, synthetic construct
  REGION 1..98: note = IGHV3-7 *01 HCVR
EVQLVESGGGLVQPGGSLRLSCAASGFTFSSYWMSWVRQAPGKGLEWVANIKQDGSEKYYVDSVKGRFTISRDNAKNSLYLQMNSLRAEDTAVYYCAR

SEQ ID NO: 75 - protein, 121 aa, synthetic construct
  REGION 1..121: note = 20H1 HCVR
EVQLVESGGGLVQPGGSLRLSCAASGFTFSTDCMGWFRQAPGKGLEGVAHIDSDGIPRYVDSVKGRFTISRDNAKNSLYLQMNSLRAEDTAVYYCVVGFKFDEDYCAPNDWGQGTMVTVSS

SEQ ID NO: 76 - protein, 121 aa, synthetic construct
  REGION 1..121: note = 20H2 HCVR
EVQLVESGGGLVQPGGSLRLSCAASGFTSRTDCMGWFRQAPGKGLEGVAHIDSDGIPRYVDSVKGRFTISRDNAKNSLYLQMNSLRAEDTAVYYCVVGFKFDEDYCAPNDWGQGTMVTVSS

SEQ ID NO: 77 - protein, 121 aa, synthetic construct
  REGION 1..121: note = 20H3 HCVR
EVQLVESGGGLVQPGGSLRLSCAASGYTFSTDCMGWFRQAPGKGLEGVAHIDSDGIPRYVDSVKGRFTISQDHAKNSLYLQMNSLRAEDTAVYYCVVGFKFDEDYCAPNDWGQGTMVTVSS

SEQ ID NO: 78 - protein, 121 aa, synthetic construct
  REGION 1..121: note = 20H4 HCVR
EVQLVESGGGLVQPGGSLRLSCAASGYTSRTDCMGWFRQAPGKGLEGVAHIDSDGIPRYVDSVKGRFTISQDHAKNSLYLQMNSLRAEDTAVYYCVVGFKFDEDYCAPNDWGQGTMVTVSS

SEQ ID NO: 79 - protein, 121 aa, synthetic construct
  REGION 1..121: note = 20H5 HCVR
EVQLVESGGGLVQPGGSLRLSCAASGYTSRTDCMGWFRQAPGKEHEGVAHIDSDGIPRYVDSVKGRFTISQDHAKNSLYLQMNSLRAEDTAVYYCVVGFKFDEDYCAPNDWGQGTMVTVSS

SEQ ID NO: 80 - protein, 120 aa, synthetic construct
  REGION 1..120: note = 30H1 HCVR
EVQLVESGGGLVQPGGSLRLSCAASGFTFSGDCMGWFRQAPGKGLEGVATIDNAGRIKYADSVKGRFTISRDNAKNSLYLQMNSLRAEDTAVYYCAAGWTFGGQCSPADWGQGTQVTVSS

SEQ ID NO: 81 - protein, 121 aa, synthetic construct
  REGION 1..121: note = 30H2 HCVR
EVQLVESGGGLVQPGGSLRLSCAASGFTFSGDCMGWFRQAPGKGLDEGVATIDNAGRIKYADSVKGRFTISRDNAKNSLYLQMNSLRAEDTAVYYCAAGWTFGGQCSPADWGQGTQVTVSS

SEQ ID NO: 82 - protein, 121 aa, synthetic construct
  REGION 1..121: note = 30H3 HCVR
EVQLVESGGGLVQPGGSLRLSCAASGYSYSGDCMGWFRQAPGKGLDEGVATIDNAGRIKYADSVKGRFTISRDNAKNSLYLQMNSLRAEDTAVYYCAAGWTFGGQCSPADWGQGTQVTVSS

SEQ ID NO: 83 - protein, 121 aa, synthetic construct
  REGION 1..121: note = 30H4 HCVR
EVQLVESGGGLVQPGGSLRLSCAASGFTFSGDCMGWFRQAPGKGLDEGVATIDNAGRIKYADSVKGRFTISHGNAKYILYLQMNSLRAEDTAVYYCAAGWTFGGQCSPADWGQGTQVTVSS

SEQ ID NO: 84 - protein, 121 aa, synthetic construct
  REGION 1..121: note = 30H5 HCVR
EVQLVESGGGLVQPGGSLRLSCAASGYSYSGDCMGWFRQAPGKGLDEGVATIDNAGRIKYADSVKGRFTISHGNAKYILYLQMNSLRAEDTAVYYCAAGWTFGGQCSPADWGQGTQVTVSS

SEQ ID NO: 85 - protein, 98 aa, synthetic construct
  REGION 1..98: note = IGHV3-30 *02
QVQLVESGGGVVQPGGSLRLSCAASGFTFSSYGMHWVRQAPGKGLEWVAFIRYDGSNKYYADSVKGRFTISRDNSKNTLYLQMNSLRAEDTAVYYCAK

SEQ ID NO: 86 - protein, 123 aa, synthetic construct
  REGION 1..123: note = 38H2 HCVR
EVQLVESGGGVVQPGGSLRLSCAASGFTFSPSDMAWFRQAPGKGLEGVATISAAGRLTYYTDSVRGRFTISRDNSKNTLYLQMNSLRAEDTAVYYCAADFAGGSSLFADYKYWGQGTMVTVSS

SEQ ID NO: 87 - protein, 123 aa, synthetic construct
  REGION 1..123: note = 38H4 HCVR
EVQLVESGGGVVQPGGSLRLSCAASPFTYGPSDMAWFRQAPGKGLEGVATISAAGRLTYYTDSVRGRFTISRDNSKNTLYLQMNSLRAEDTAVYYCAADFAGGSSLFADYKYWGQGTMVTVSS

SEQ ID NO: 88 - protein, 123 aa, synthetic construct
  REGION 1..123: note = 38H7 HCVR
EVQLVESGGGVVQPGGSLRLSCAASPSTYGPSDMAWFRQAPGKQREGVATISAAGRLTYYTDSVRGRFTISRDNSKNTMYLQMNSLRAEDTAVYYCAADFAGGSSLFADYKYWGQGTMVTVSS

SEQ ID NO: 89 - protein, 123 aa, synthetic construct
  REGION 1..123: note = 38H8 HCVR
EVQLVESGGGVVQPGGSLRLSCAASPSTYGPSDMAWFRQAPGKGLEGVATISAAGRLTYYTDSVRGRFTISRDNSKNTLYLQMNSLRAEDTAVYYCAADFAGGSSLFADYKYWGQGTMVTVSS

SEQ ID NO: 90 - protein, 123 aa, synthetic construct
  REGION 1..123: note = 38H9 HCVR
EVQLVESGGGVVQPGGSLRLSCAASPSTYGPSDMAWFRQAPGKGLEGVATISAAGRLTYYTDSVRGRFTISRDNSKNTMYLQMNSLRAEDTAVYYCAADFAGGSSLFADYKYWGQGTMVTVSS

SEQ ID NO: 91 - protein, 120 aa, synthetic construct
  REGION 1..120: note = 39H1 HCVR
EVQLVESGGGLVQPGGSLRLSCAASGFTFSTDCMGWFRQAPGKGLEGVAHIDSDGIPRYVESVKGRFTISRDNAKNSLYLQMNSLRAEDTAVYYCVVGFKFGDYCAPNDWGQGTMVTVSS

SEQ ID NO: 92 - protein, 120 aa, synthetic construct
  REGION 1..120: note = 39H2 HCVR
EVQLVESGGGLVQPGGSLRLSCAASGFTSRTDCMGWFRQAPGKGLEGVAHIDSDGIPRYVESVKGRFTISRDNAKNSLYLQMNSLRAEDTAVYYCVVGFKFGDYCAPNDWGQGTMVTVSS

SEQ ID NO: 93 - protein, 120 aa, synthetic construct
  REGION 1..120: note = 39H3 HCVR
EVQLVESGGGLVQPGGSLRLSCAASGYTFSTDCMGWFRQAPGKGLEGVAHIDSDGIPRYVESVKGRFTISQDHAKNSLYLQMNSLRAEDTAVYYCVVGFKFGDYCAPNDWGQGTMVTVSS

SEQ ID NO: 94 - protein, 120 aa, synthetic construct
  REGION 1..120: note = 39H4 HCVR
EVQLVESGGGLVQPGGSLRLSCAASGYTSRTDCMGWFRQAPGKGLEGVAHIDSDGIPRYVESVKGRFTISQDHAKNSLYLQMNSLRAEDTAVYYCVVGFKFGDYCAPNDWGQGTMVTVSS

SEQ ID NO: 95 - protein, 120 aa, synthetic construct
  REGION 1..120: note = 39H5 HCVR
EVQLVESGGGLVQPGGSLRLSCAASGYTSRTDCMGWFRQAPGKEREGVAHIDSDGIPRYVESVKGRFTISQDHAKNSLYLQMNSLRAEDTAVYYCVVGFKFGDYCAPNDWGQGTMVTVSS

SEQ ID NO: 96 - protein, 125 aa, synthetic construct
  REGION 1..125: note = 151H2 HCVR
EVQLVESGGGLVQPGGSLRLSCAASGFTYRPYCMAWFRQAPGKGLEAVAGIDIFGGTTYADSVKGRFTISRDNAKNSLYLQMNSLRAEDTAVYYCAAGDSPDGRCPPLGQGLNYWGQGTMVTVSS

SEQ ID NO: 97 - protein, 127 aa, synthetic construct
  REGION 1..127: note = 151H4 HCVR
EVQLVESGGGLVQPGGSLRLSCVASASGFTYRPYCMAWFRQAPGKGLEAVAGIDIFGGTTYADSVKGRFTISRDNAKNSLYLQMNSLRAEDTAVYYCAAGDSPDGRCPPLGQGLNYWGQGTMVTVSS

SEQ ID NO: 98 - protein, 127 aa, synthetic construct
  REGION 1..127: note = 151H7 HCVR
HVQLVESGGGLVQPGGSLRLSCVASASGFTYRPYCMAWFRQAPGKEREAVAGIDIFGGTTYADSVKGRFTASRDNAGFSLYLQMNSLRAEDTAVYYCAAGDSPDGRCPPLGQGLNYWGQGTMVTVSS

SEQ ID NO: 99 - protein, 127 aa, synthetic construct
  REGION 1..127: note = 151H8 HCVR
EVQLVESGGGLVQPGGSLRLSCVASASGFTYRPYCMAWFRQAPGKGLEAVAGIDIFGGTTYADSVKGRFTISRDNAGFSLYLQMNSLRAEDTAVYYCAAGDSPDGRCPPLGQGLNYWGQGTMVTVSS

SEQ ID NO: 100 - protein, 127 aa, synthetic construct
  REGION 1..127: note = 151H9 HCVR
HVQLVESGGGLVQPGGSLRLSCVASASGFTYRPYCMAWFRQAPGKGLEAVAGIDIFGGTTYADSVKGRFTASRDNAGFSLYLQMNSLRAEDTAVYYCAAGDSPDGRCPPLGQGLNYWGQGTMVTVSS

SEQ ID NO: 101 - protein, 229 aa, synthetic construct
  REGION 1..229: note = IgG4FcS228P/F234A/L235A/K447A
ESKYGPPCPPCPAPEAAGGPSVFLFPPKPKDTLMISRTPEVTCVVVDVSQEDPEVQFNWYVDGVEVHNAKTKPREEQFNSTYRVVSVLTVLHQDWLNGKEYKCKVSNKGLPSSIEKTISKAKGQPREPQVYTLPPSQEEMTKNQVSLTCLVKGFYPSDIAVEWESNGQPENNYKTTPPVLDSDGSFFLYSRLTVDKSRWQEGNVFSCSVMHEALHNHYTQKSLSLSLGA

SEQ ID NO: 102 - protein, 446 aa, synthetic construct
  REGION 1..446: note = 1708TIGITHC
EVQLVQSGAEVKKPGASVKVSCKASGYTFTNYWMHWVRQAPGQGLEWMGRIDPDSTGSKYNEKFKTRVTMTRDTSTSTVYMELSSLRSEDTAVYYCAREGAYGYYFDYWGQGTLVTVSSASTKGPSVFPLAPCSRSTSESTAALGCLVKDYFPEPVTVSWNSGALTSGVHTFPAVLQSSGLYSLSSVVTVPSSSLGTKTYTCNVDHKPSNTKVDKRVESKYGPPCPPCPAPEFLGGPSVFLFPPKPKDTLMISRTPEVTCVVVDVSQEDPEVQFNWYVDGVEVHNAKTKPREEQFNSTYRVVSVLTVLHQDWLNGKEYKCKVSNKGLPSSIEKTISKAKGQPREPQVYTLPPSQEEMTKNQVSLTCLVKGFYPSDIAVEWESNGQPENNYKTTPPVLDSDGSFFLYSRLTVDKSRWQEGNVFSCSVMHEALHNHYTQKSLSLSLGK

SEQ ID NO: 103 - protein, 214 aa, synthetic construct
  REGION 1..214: note = 1708TIGIT LC
DIQMTQSPSSLSASVGDRVTITCRASENIYSYLAWYQQKPGKSPKLLIYNARTLAEGVPSRFSGSGSGTDFTLTISSLQPEDFATYYCQYHSGSPLPFGGGTKVEIKRTVAAPSVFIFPPSDEQLKSGTASVVCLLNNFYPREAKVQWKVDNALQSGNSQESVTEQDSKDSTYSLSSTLTLSKADYEKHKVYACEVTHQGLSSPVTKSFNRGEC

SEQ ID NO: 104 - protein, 583 aa, synthetic construct
  REGION 1..583: note = 1708-151-11511708N
HVQLVESGGGSVQAGGSLRLSCVASASGFTYRPYCMAWFRQAPGKEREAVAGIDIFGGTTYADSVKGRFTASRDNAGFSLFLQMNDLKPEDTAMYYCAAGDSPDGRCPPLGQGLNYWGQGTQVTVSSGGGGSGGGGSEVQLVQSGAEVKKPGASVKVSCKASGYTFTNYWMHWVRQAPGQGLEWMGRIDPDSTGSKYNEKFKTRVTMTRDTSTSTVYMELSSLRSEDTAVYYCAREGAYGYYFDYWGQGTLVTVSSASTKGPSVFPLAPCSRSTSESTAALGCLVKDYFPEPVTVSWNSGALTSGVHTFPAVLQSSGLYSLSSVVTVPSSSLGTKTYTCNVDHKPSNTKVDKRVESKYGPPCPPCPAPEFLGGPSVFLFPPKPKDTLMISRTPEVTCVVVDVSQEDPEVQFNWYVDGVEVHNAKTKPREEQFNSTYRVVSVLTVLHQDWLNGKEYKCKVSNKGLPSSIEKTISKAKGQPREPQVYTLPPSQEEMTKNQVSLTCLVKGFYPSDIAVEWESNGQPENNYKTTPPVLDSDGSFFLYSRLTVDKSRWQEGNVFSCSVMHEALHNHYTQKSLSLSLGK

SEQ ID NO: 105 - protein, 583 aa, synthetic construct
  REGION 1..583: note = 1708-151-21511708C
EVQLVQSGAEVKKPGASVKVSCKASGYTFTNYWMHWVRQAPGQGLEWMGRIDPDSTGSKYNEKFKTRVTMTRDTSTSTVYMELSSLRSEDTAVYYCAREGAYGYYFDYWGQGTLVTVSSASTKGPSVFPLAPCSRSTSESTAALGCLVKDYFPEPVTVSWNSGALTSGVHTFPAVLQSSGLYSLSSVVTVPSSSLGTKTYTCNVDHKPSNTKVDKRVESKYGPPCPPCPAPEFLGGPSVFLFPPKPKDTLMISRTPEVTCVVVDVSQEDPEVQFNWYVDGVEVHNAKTKPREEQFNSTYRVVSVLTVLHQDWLNGKEYKCKVSNKGLPSSIEKTISKAKGQPREPQVYTLPPSQEEMTKNQVSLTCLVKGFYPSDIAVEWESNGQPENNYKTTPPVLDSDGSFFLYSRLTVDKSRWQEGNVFSCSVMHEALHNHYTQKSLSLSLGKGGGGSGGGGSHVQLVESGGGSVQAGGSLRLSCVASASGFTYRPYCMAWFRQAPGKEREAVAGIDIFGGTTYADSVKGRFTASRDNAGFSLFLQMNDLKPEDTAMYYCAAGDSPDGRCPPLGQGLNYWGQGTQVTVSS

SEQ ID NO: 106 - protein, 351 aa, synthetic construct
  REGION 1..351: note = 1708-151-31511708N
HVQLVESGGGSVQAGGSLRLSCVASASGFTYRPYCMAWFRQAPGKEREAVAGIDIFGGTTYADSVKGRFTASRDNAGFSLFLQMNDLKPEDTAMYYCAAGDSPDGRCPPLGQGLNYWGQGTQVTVSSGGGGSGGGGSDIQMTQSPSSLSASVGDRVTITCRASENIYSYLAWYQQKPGKSPKLLIYNARTLAEGVPSRFSGSGSGTDFTLTISSLQPEDFATYYCQYHSGSPLPFGGGTKVEIKRTVAAPSVFIFPPSDEQLKSGTASVVCLLNNFYPREAKVQWKVDNALQSGNSQESVTEQDSKDSTYSLSSTLTLSKADYEKHKVYACEVTHQGLSSPVTKSFNRGEC

SEQ ID NO: 107 - protein, 351 aa, synthetic construct
  REGION 1..351: note = 1708-151-41511708C
DIQMTQSPSSLSASVGDRVTITCRASENIYSYLAWYQQKPGKSPKLLIYNARTLAEGVPSRFSGSGSGTDFTLTISSLQPEDFATYYCQYHSGSPLPFGGGTKVEIKRTVAAPSVFIFPPSDEQLKSGTASVVCLLNNFYPREAKVQWKVDNALQSGNSQESVTEQDSKDSTYSLSSTLTLSKADYEKHKVYACEVTHQGLSSPVTKSFNRGECGGGGSGGGGSHVQLVESGGGSVQAGGSLRLSCVASASGFTYRPYCMAWFRQAPGKEREAVAGIDIFGGTTYADSVKGRFTASRDNAGFSLFLQMNDLKPEDTAMYYCAAGDSPDGRCPPLGQGLNYWGQGTQVTVSS

SEQ ID NO: 108 - protein, 577 aa, synthetic construct
  REGION 1..577: note = 1708-20H5
EVQLVESGGGLVQPGGSLRLSCAASGYTSRTDCMGWFRQAPGKEHEGVAHIDSDGIPRYVDSVKGRFTISQDHAKNSLYLQMNSLRAEDTAVYYCVVGFKFDEDYCAPNDWGQGTMVTVSSGGGGSGGGGSEVQLVQSGAEVKKPGASVKVSCKASGYTFTNYWMHWVRQAPGQGLEWMGRIDPDSTGSKYNEKFKTRVTMTRDTSTSTVYMELSSLRSEDTAVYYCAREGAYGYYFDYWGQGTLVTVSSASTKGPSVFPLAPCSRSTSESTAALGCLVKDYFPEPVTVSWNSGALTSGVHTFPAVLQSSGLYSLSSVVTVPSSSLGTKTYTCNVDHKPSNTKVDKRVESKYGPPCPPCPAPEFLGGPSVFLFPPKPKDTLMISRTPEVTCVVVDVSQEDPEVQFNWYVDGVEVHNAKTKPREEQFNSTYRVVSVLTVLHQDWLNGKEYKCKVSNKGLPSSIEKTISKAKGQPREPQVYTLPPSQEEMTKNQVSLTCLVKGFYPSDIAVEWESNGQPENNYKTTPPVLDSDGSFFLYSRLTVDKSRWQEGNVFSCSVMHEALHNHYTQKSLSLSLGK

SEQ ID NO: 109 - protein, 577 aa, synthetic construct
  REGION 1..577: note = 1708-30H2
EVQLVESGGGLVQPGGSLRLSCAASGFTFSGDCMGWFRQAPGKGLDEGVATIDNAGRIKYADSVKGRFTISRDNAKNSLYLQMNSLRAEDTAVYYCAAGWTFGGQCSPADWGQGTQVTVSSGGGGSGGGGSEVQLVQSGAEVKKPGASVKVSCKASGYTFTNYWMHWVRQAPGQGLEWMGRIDPDSTGSKYNEKFKTRVTMTRDTSTSTVYMELSSLRSEDTAVYYCAREGAYGYYFDYWGQGTLVTVSSASTKGPSVFPLAPCSRSTSESTAALGCLVKDYFPEPVTVSWNSGALTSGVHTFPAVLQSSGLYSLSSVVTVPSSSLGTKTYTCNVDHKPSNTKVDKRVESKYGPPCPPCPAPEFLGGPSVFLFPPKPKDTLMISRTPEVTCVVVDVSQEDPEVQFNWYVDGVEVHNAKTKPREEQFNSTYRVVSVLTVLHQDWLNGKEYKCKVSNKGLPSSIEKTISKAKGQPREPQVYTLPPSQEEMTKNQVSLTCLVKGFYPSDIAVEWESNGQPENNYKTTPPVLDSDGSFFLYSRLTVDKSRWQEGNVFSCSVMHEALHNHYTQKSLSLSLGK

SEQ ID NO: 110 - protein, 576 aa, synthetic construct
  REGION 1..576: note = 1708-39H2
EVQLVESGGGLVQPGGSLRLSCAASGFTSRTDCMGWFRQAPGKGLEGVAHIDSDGIPRYVESVKGRFTISRDNAKNSLYLQMNSLRAEDTAVYYCVVGFKFGDYCAPNDWGQGTMVTVSSGGGGSGGGGSEVQLVQSGAEVKKPGASVKVSCKASGYTFTNYWMHWVRQAPGQGLEWMGRIDPDSTGSKYNEKFKTRVTMTRDTSTSTVYMELSSLRSEDTAVYYCAREGAYGYYFDYWGQGTLVTVSSASTKGPSVFPLAPCSRSTSESTAALGCLVKDYFPEPVTVSWNSGALTSGVHTFPAVLQSSGLYSLSSVVTVPSSSLGTKTYTCNVDHKPSNTKVDKRVESKYGPPCPPCPAPEFLGGPSVFLFPPKPKDTLMISRTPEVTCVVVDVSQEDPEVQFNWYVDGVEVHNAKTKPREEQFNSTYRVVSVLTVLHQDWLNGKEYKCKVSNKGLPSSIEKTISKAKGQPREPQVYTLPPSQEEMTKNQVSLTCLVKGFYPSDIAVEWESNGQPENNYKTTPPVLDSDGSFFLYSRLTVDKSRWQEGNVFSCSVMHEALHNHYTQKSLSLSLGK

SEQ ID NO: 111 - protein, 583 aa, synthetic construct
  REGION 1..583: note = 1708-151H7
HVQLVESGGGLVQPGGSLRLSCVASASGFTYRPYCMAWFRQAPGKEREAVAGIDIFGGTTYADSVKGRFTASRDNAGFSLYLQMNSLRAEDTAVYYCAAGDSPDGRCPPLGQGLNYWGQGTMVTVSSGGGGSGGGGSEVQLVQSGAEVKKPGASVKVSCKASGYTFTNYWMHWVRQAPGQGLEWMGRIDPDSTGSKYNEKFKTRVTMTRDTSTSTVYMELSSLRSEDTAVYYCAREGAYGYYFDYWGQGTLVTVSSASTKGPSVFPLAPCSRSTSESTAALGCLVKDYFPEPVTVSWNSGALTSGVHTFPAVLQSSGLYSLSSVVTVPSSSLGTKTYTCNVDHKPSNTKVDKRVESKYGPPCPPCPAPEFLGGPSVFLFPPKPKDTLMISRTPEVTCVVVDVSQEDPEVQFNWYVDGVEVHNAKTKPREEQFNSTYRVVSVLTVLHQDWLNGKEYKCKVSNKGLPSSIEKTISKAKGQPREPQVYTLPPSQEEMTKNQVSLTCLVKGFYPSDIAVEWESNGQPENNYKTTPPVLDSDGSFFLYSRLTVDKSRWQEGNVFSCSVMHEALHNHYTQKSLSLSLGK

SEQ ID NO: 112 - protein, 583 aa, synthetic construct
  REGION 1..583: note = 1708-151H8
EVQLVESGGGLVQPGGSLRLSCVASASGFTYRPYCMAWFRQAPGKGLEAVAGIDIFGGTTYADSVKGRFTISRDNAGFSLYLQMNSLRAEDTAVYYCAAGDSPDGRCPPLGQGLNYWGQGTMVTVSSGGGGSGGGGSEVQLVQSGAEVKKPGASVKVSCKASGYTFTNYWMHWVRQAPGQGLEWMGRIDPDSTGSKYNEKFKTRVTMTRDTSTSTVYMELSSLRSEDTAVYYCAREGAYGYYFDYWGQGTLVTVSSASTKGPSVFPLAPCSRSTSESTAALGCLVKDYFPEPVTVSWNSGALTSGVHTFPAVLQSSGLYSLSSVVTVPSSSLGTKTYTCNVDHKPSNTKVDKRVESKYGPPCPPCPAPEFLGGPSVFLFPPKPKDTLMISRTPEVTCVVVDVSQEDPEVQFNWYVDGVEVHNAKTKPREEQFNSTYRVVSVLTVLHQDWLNGKEYKCKVSNKGLPSSIEKTISKAKGQPREPQVYTLPPSQEEMTKNQVSLTCLVKGFYPSDIAVEWESNGQPENNYKTTPPVLDSDGSFFLYSRLTVDKSRWQEGNVFSCSVMHEALHNHYTQKSLSLSLGK

SEQ ID NO: 113 - protein, 449 aa, synthetic construct
  REGION 1..449: note = 1708-IgG1 (1708IgG1) HC
EVQLVQSGAEVKKPGASVKVSCKASGYTFTNYWMHWVRQAPGQGLEWMGRIDPDSTGSKYNEKFKTRVTMTRDTSTSTVYMELSSLRSEDTAVYYCAREGAYGYYFDYWGQGTLVTVSSASTKGPSVFPLAPSSKSTSGGTAALGCLVKDYFPEPVTVSWNSGALTSGVHTFPAVLQSSGLYSLSSVVTVPSSSLGTQTYICNVNHKPSNTKVDKKVEPKSCDKTHTCPPCPAPELLGGPSVFLFPPKPKDTLMISRTPEVTCVVVDVSHEDPEVKFNWYVDGVEVHNAKTKPREEQYNSTYRVVSVLTVLHQDWLNGKEYKCKVSNKALPAPIEKTISKAKGQPREPQVYTLPPSREEMTKNQVSLTCLVKGFYPSDIAVEWESNGQPENNYKTTPPVLDSDGSFFLYSKLTVDKSRWQQGNVFSCSVMHEALHNHYTQKSLSLSPGK

SEQ ID NO: 114 - protein, 586 aa, synthetic construct
  REGION 1..586: note = 1708-151-IgG1 (1708-151IgG1)
HVQLVESGGGSVQAGGSLRLSCVASASGFTYRPYCMAWFRQAPGKEREAVAGIDIFGGTTYADSVKGRFTASRDNAGFSLFLQMNDLKPEDTAMYYCAAGDSPDGRCPPLGQGLNYWGQGTQVTVSSGGGGSGGGGSEVQLVQSGAEVKKPGASVKVSCKASGYTFTNYWMHWVRQAPGQGLEWMGRIDPDSTGSKYNEKFKTRVTMTRDTSTSTVYMELSSLRSEDTAVYYCAREGAYGYYFDYWGQGTLVTVSSASTKGPSVFPLAPSSKSTSGGTAALGCLVKDYFPEPVTVSWNSGALTSGVHTFPAVLQSSGLYSLSSVVTVPSSSLGTQTYICNVNHKPSNTKVDKKVEPKSCDKTHTCPPCPAPELLGGPSVFLFPPKPKDTLMISRTPEVTCVVVDVSHEDPEVKFNWYVDGVEVHNAKTKPREEQYNSTYRVVSVLTVLHQDWLNGKEYKCKVSNKALPAPIEKTISKAKGQPREPQVYTLPPSREEMTKNQVSLTCLVKGFYPSDIAVEWESNGQPENNYKTTPPVLDSDGSFFLYSKLTVDKSRWQQGNVFSCSVMHEALHNHYTQKSLSLSPGK

SEQ ID NO: 115 - protein, 5 aa, synthetic construct
  REGION 1..5: note = 1707 HCDR1
DYHMY

SEQ ID NO: 116 - protein, 17 aa, synthetic construct
  REGION 1..17: note = 1707 HCDR2
YISKGGISTYYPDTVKG

SEQ ID NO: 117 - protein, 10 aa, synthetic construct
  REGION 1..10: note = 1707 HCDR3
QSSYDFAMDY

SEQ ID NO: 118 - protein, 11 aa, synthetic construct
  REGION 1..11: note = 1707 LCDR1
KASQDVGTSVA

SEQ ID NO: 119 - protein, 7 aa, synthetic construct
  REGION 1..7: note = 1707 LCDR2
WASARHT

SEQ ID NO: 120 - protein, 9 aa, synthetic construct
  REGION 1..9: note = 1707 LCDR3
QQYSSYPLT

SEQ ID NO: 121 - protein, 5 aa, synthetic construct
  REGION 1..5: note = 1708 HCDR1
NYWMH

SEQ ID NO: 122 - protein, 17 aa, synthetic construct
  REGION 1..17: note = 1708 HCDR2
RIDPDSTGSKYNEKFKT

SEQ ID NO: 123 - protein, 10 aa, synthetic construct
  REGION 1..10: note = 1708 HCDR3
EGAYGYYFDY

SEQ ID NO: 124 - protein, 11 aa, synthetic construct
  REGION 1..11: note = 1708 LCDR1
RASENIYSYLA

SEQ ID NO: 125 - protein, 7 aa, synthetic construct
  REGION 1..7: note = 1708 LCDR2
NARTLAE

SEQ ID NO: 126 - protein, 9 aa, synthetic construct
  REGION 1..9: note = 1708 LCDR3
QYHSGSPLP

SEQ ID NO: 127 - protein, 5 aa, synthetic construct
  REGION 1..5: note = 1709 HCDR1
DYYMH

SEQ ID NO: 128 - protein, 17 aa, synthetic construct
  REGION 1..17: note = 1709 HCDR2
LVYPYNDNTGYNRKFKG

SEQ ID NO: 129 - protein, 11 aa, synthetic construct
  REGION 1..11: note = 1709 HCDR3
GGPSNWNYFDY

SEQ ID NO: 130 - protein, 11 aa, synthetic construct
  REGION 1..11: note = 1709 LCDR1
KASQNVVTAVA

SEQ ID NO: 131 - protein, 7 aa, synthetic construct
  REGION 1..7: note = 1709 LCDR2
SASNRYT

SEQ ID NO: 132 - protein, 9 aa, synthetic construct
  REGION 1..9: note = 1709 HCDR3
QQYTLYPLT

SEQ ID NO: 133 - protein, 5 aa, synthetic construct
  REGION 1..5: note = 1710 HCDR1
NYYMH

SEQ ID NO: 134 - protein, 17 aa, synthetic construct
  REGION 1..17: note = 1710 HCDR2
RIDPTSGATKYNDNFKG

SEQ ID NO: 135 - protein, 10 aa, synthetic construct
  REGION 1..10: note = 1710 HCDR3
EGGFGYYFDY

SEQ ID NO: 136 - protein, 11 aa, synthetic construct
  REGION 1..11: note = 1710 LCDR1
RTSENIFTYLA

SEQ ID NO: 137 - protein, 7 aa, synthetic construct
  REGION 1..7: note = 1710 LCDR2
NAKTFAE

SEQ ID NO: 138 - protein, 9 aa, synthetic construct
  REGION 1..9: note = 1710 LCDR3
QHHYGIPLP

SEQ ID NO: 139 - protein, 5 aa, synthetic construct
  REGION 1..5: note = 1711 HCDR1
NYWIG

SEQ ID NO: 140 - protein, 17 aa, synthetic construct
  REGION 1..17: note = 1711 HCDR2
DIYPGGAYTNYNEKFKD

SEQ ID NO: 141 - protein, 13 aa, synthetic construct
  REGION 1..13: note = 1711 HCDR3
GDYYDSSGRAMDY

SEQ ID NO: 142 - protein, 17 aa, synthetic construct
  REGION 1..17: note = 1711 LCDR1
KSSQSLLYSRNQMNYLA

SEQ ID NO: 143 - protein, 7 aa, synthetic construct
  REGION 1..7: note = 1711 LCDR2
WTSTRES

SEQ ID NO: 144 - protein, 9 aa, synthetic construct
  REGION 1..9: note = 1711 LCDR3
QQYYSYPYT

SEQ ID NO: 145 - protein, 119 aa, synthetic construct
  REGION 1..119: note = 1708-VH1
EVQLVQSGAEVKKPGASVKVSCKASGYTFTNYWMHWVRQAPGQGLEWMGRIDPDSTGSKYNEKFKTRVTMTRDTSTSTVYMELSSLRSEDTAVYYCAREGAYGYYFDYWGQGTLVTVSS

SEQ ID NO: 146 - protein, 119 aa, synthetic construct
  REGION 1..119: note = 1708-VH2
EVQLVQSGAEVKKPGASVKVSCKASGYTFTNYWMHWVRQAPGQGLEWMGRIDPDSTGSKYNEKFKTRVTMTVDTSTSTVYMELSSLRSEDTAVYYCAREGAYGYYFDYWGQGTLVTVSS

SEQ ID NO: 147 - protein, 119 aa, synthetic construct
  REGION 1..119: note = 1708-VH3
EVQLVQSGAEVKKPGASVKVSCKASGYTFTNYWMHWVRQAPGQGLEWIGRIDPDSTGSKYNEKFKTRVTMTVDTSTSTAYMELSSLRSEDTAVYYCAREGAYGYYFDYWGQGTLVTVSS

SEQ ID NO: 148 - protein, 107 aa, synthetic construct
  REGION 1..107: note = 1708-VL1
DIQMTQSPSSLSASVGDRVTITCRASENIYSYLAWYQQKPGKAPKLLIYNARTLAEGVPSRFSGSGSGTDFTLTISSLQPEDFATYYCQYHSGSPLPFGGGTKVEIK

SEQ ID NO: 149 - protein, 107 aa, synthetic construct
  REGION 1..107: note = 1708-VL2
DIQMTQSPSSLSASVGDRVTITCRASENIYSYLAWYQQKPGKSPKLLIYNARTLAEGVPSRFSGSGSGTDFTLTISSLQPEDFATYYCQYHSGSPLPFGGGTKVEIK

SEQ ID NO: 150 - protein, 13 aa, synthetic construct
  REGION 1..13: note = 20 HCDR3
GFKFDEDYCAPND

SEQ ID NO: 151 - protein, 12 aa, synthetic construct
  REGION 1..12: note = 30 HCDR3
GWTFGGQCSPAD

SEQ ID NO: 152 - protein, 10 aa, synthetic construct
  REGION 1..10: note = LINKER
GGGGSGGGGS

SEQ ID NO: 153 - protein, 229 aa, synthetic construct
  REGION 1..229: note = IgG4FcS228P/K447A
ESKYGPPCPPCPAPEFLGGPSVFLFPPKPKDTLMISRTPEVTCVVVDVSQEDPEVQFNWYVDGVEVHNAKTKPREEQFNSTYRVVSVLTVLHQDWLNGKEYKCKVSNKGLPSSIEKTISKAKGQPREPQVYTLPPSQEEMTKNQVSLTCLVKGFYPSDIAVEWESNGQPENNYKTTPPVLDSDGSFFLYSRLTVDKSRWQEGNVFSCSVMHEALHNHYTQKSLSLSLGK

SEQ ID NO: 154 - protein, 4 aa, synthetic construct
ASGS

SEQ ID NO: 155 - protein, 5 aa, synthetic construct
GGGGS

SEQ ID NO: 156 - protein, 15 aa, synthetic construct
GGGGSGGGGSGGGGS

SEQ ID NO: 157 - protein, 20 aa, synthetic construct
GGGGSGGGGSGGGGSGGGGS

SEQ ID NO: 158 - protein, 25 aa, synthetic construct
GGGGSGGGGSGGGGSGGGGSGGGGS

SEQ ID NO: 159 - protein, 30 aa, synthetic construct
GGGGSGGGGSGGGGSGGGGSGGGGSGGGGS

SEQ ID NO: 160 - protein, 5 aa, synthetic construct
YGNGT

SEQ ID NO: 161 - protein, 10 aa, synthetic construct
YGNGTYGNGT

SEQ ID NO: 162 - protein, 15 aa, synthetic construct
YGNGTYGNGTYGNGT

SEQ ID NO: 163 - protein, 20 aa, synthetic construct
YGNGTYGNGTYGNGTYGNGT

SEQ ID NO: 164 - protein, 25 aa, synthetic construct
YGNGTYGNGTYGNGTYGNGTYGNGT

SEQ ID NO: 165 - protein, 30 aa, synthetic construct
YGNGTYGNGTYGNGTYGNGTYGNGTYGNGT